European Patent Specification EP 2 970 416 B1, published November 22, 2023. Title: METHODS FOR TREATMENT OF NEPHROTIC SYNDROME AND RELATED CONDITIONS. Applicant: The UAB Research Foundation Chugh, Sumant  S. The sequence listing filed with the application follows.

SEQUENCE LISTING (94 sequences)

SEQ ID NO: 1 - protein, 406 aa, Homo sapiens
MSGAPTAGAALMLCAATAVLLSAQGGPVQSKSPRFASWDEMNVLAHGLLQLGQGLREHAERTRSQLSALERRLSACGSACQGTEGSTDLPLAPESRVDPEVLHSLQTQLKAQNSRIQQLFHKVAQQQRHLEKQHLRIQHLQSQFGLLDHKHLDHEVAKPARRKRLPEMAQPVDPAHNVSRLHRLPRDCQELFQVGERQSGLFEIQPQGSPPFLVNCKMTSDGGWTVIQRRHDGSVDFNRPWEAYKAGFGDPHGEFWLGLEKVHSITGDRNSRLAVQLRDWDGNAELLQFSVHLGGEDTAYSLQLTAPVAGQLGATTVPPSGLSVPFSTWDQDHDLRRDKNCAKSLSGGWWFGTCSHSNLNGQYFRSIPQQRQKLKKGIFWKTWRGRYYPLQATTMLIQPMAAEAAS

SEQ ID NO: 2 - DNA, 1967 bp, Homo sapiens
ataaaaaccgtcctcgggcgcggcggggagaagccgagctgagcggatcctcacacgactgtgatccgattctttccagcggcttctgcaaccaagcgggtcttacccccggtcctccgcgtctccagtcctcgcacctggaaccccaacgtccccgagagtccccgaatccccgctcccaggctacctaagaggatgagcggtgctccgacggccggggcagccctgatgctctgcgccgccaccgccgtgctactgagcgctcagggcggacccgtgcagtccaagtcgccgcgctttgcgtcctgggacgagatgaatgtcctggcgcacggactcctgcagctcggccaggggctgcgcgaacacgcggagcgcacccgcagtcagctgagcgcgctggagcggcgcctgagcgcgtgcgggtccgcctgtcagggaaccgaggggtccaccgacctcccgttagcccctgagagccgggtggaccctgaggtccttcacagcctgcagacacaactcaaggctcagaacagcaggatccagcaactcttccacaaggtggcccagcagcagcggcacctggagaagcagcacctgcgaattcagcatctgcaaagccagtttggcctcctggaccacaagcacctagaccatgaggtggccaagcctgcccgaagaaagaggctgcccgagatggcccagccagttgacccggctcacaatgtcagccgcctgcaccggctgcccagggattgccaggagctgttccaggttggggagaggcagagtggactatttgaaatccagcctcaggggtctccgccatttttggtgaactgcaagatgacctcagatggaggctggacagtaattcagaggcgccacgatggctcagtggacttcaaccggccctgggaagcctacaaggcggggtttggggatccccacggcgagttctggctgggtctggagaaggtgcatagcatcacgggggaccgcaacagccgcctggccgtgcagctgcgggactgggatggcaacgccgagttgctgcagttctccgtgcacctgggtggcgaggacacggcctatagcctgcagctcactgcacccgtggccggccagctgggcgccaccaccgtcccacccagcggcctctccgtacccttctccacttgggaccaggatcacgacctccgcagggacaagaactgcgccaagagcctctctggaggctggtggtttggcacctgcagccattccaacctcaacggccagtacttccgctccatcccacagcagcggcagaagcttaagaagggaatcttctggaagacctggcggggccgctactacccgctgcaggccaccaccatgttgatccagcccatggcagcagaggcagcctcctagcgtcctggctgggcctggtcccaggcccacgaaagacggtgactcttggctctgcccgaggatgtggccgttccctgcctgggcaggggctccaaggaggggccatctggaaacttgtggacagagaagaagaccacgactggagaagccccctttctgagtgcaggggggctgcatgcgttgcctcctgagatcgaggctgcaggatatgctcagactctagaggcgtggaccaaggggcatggagcttcactccttgctggccagggagttggggactcagagggaccacttggggccagccagactggcctcaatggcggactcagtcacattgactgacggggaccagggcttgtgtgggtcgagagcgccctcatggtgctggtgctgttgtgtgtaggtcccctggggacacaagcaggcgccaatggtatctgggcggagctcacagagttcttggaataaaagcaacctcagaacacttaaaaaaaaaaaaaaaaaaaaaaaaaaaaaaaaaaaaaaaaaaaaaaaaaaaaaaaaaaaaaaaa

SEQ ID NO: 3 - protein, 368 aa, Homo sapiens
MSGAPTAGAALMLCAATAVLLSAQGGPVQSKSPRFASWDEMNVLAHGLLQLGQGLREHAERTRSQLSALERRLSACGSACQGTEGSTDLPLAPESRVDPEVLHSLQTQLKAQNSRIQQLFHKVAQQQRHLEKQHLRIQHLQSQFGLLDHKHLDHEVAKPARRKRLPEMAQPVDPAHNVSRLHHGGWTVIQRRHDGSVDFNRPWEAYKAGFGDPHGEFWLGLEKVHSITGDRNSRLAVQLRDWDGNAELLQFSVHLGGEDTAYSLQLTAPVAGQLGATTVPPSGLSVPFSTWDQDHDLRRDKNCAKSLSGGWWFGTCSHSNLNGQYFRSIPQQRQKLKKGIFWKTWRGRYYPLQATTMLIQPMAAEAAS

SEQ ID NO: 4 - DNA, 1853 bp, Homo sapiens
ataaaaaccgtcctcgggcgcggcggggagaagccgagctgagcggatcctcacacgactgtgatccgattctttccagcggcttctgcaaccaagcgggtcttacccccggtcctccgcgtctccagtcctcgcacctggaaccccaacgtccccgagagtccccgaatccccgctcccaggctacctaagaggatgagcggtgctccgacggccggggcagccctgatgctctgcgccgccaccgccgtgctactgagcgctcagggcggacccgtgcagtccaagtcgccgcgctttgcgtcctgggacgagatgaatgtcctggcgcacggactcctgcagctcggccaggggctgcgcgaacacgcggagcgcacccgcagtcagctgagcgcgctggagcggcgcctgagcgcgtgcgggtccgcctgtcagggaaccgaggggtccaccgacctcccgttagcccctgagagccgggtggaccctgaggtccttcacagcctgcagacacaactcaaggctcagaacagcaggatccagcaactcttccacaaggtggcccagcagcagcggcacctggagaagcagcacctgcgaattcagcatctgcaaagccagtttggcctcctggaccacaagcacctagaccatgaggtggccaagcctgcccgaagaaagaggctgcccgagatggcccagccagttgacccggctcacaatgtcagccgcctgcaccatggaggctggacagtaattcagaggcgccacgatggctcagtggacttcaaccggccctgggaagcctacaaggcggggtttggggatccccacggcgagttctggctgggtctggagaaggtgcatagcatcacgggggaccgcaacagccgcctggccgtgcagctgcgggactgggatggcaacgccgagttgctgcagttctccgtgcacctgggtggcgaggacacggcctatagcctgcagctcactgcacccgtggccggccagctgggcgccaccaccgtcccacccagcggcctctccgtacccttctccacttgggaccaggatcacgacctccgcagggacaagaactgcgccaagagcctctctggaggctggtggtttggcacctgcagccattccaacctcaacggccagtacttccgctccatcccacagcagcggcagaagcttaagaagggaatcttctggaagacctggcggggccgctactacccgctgcaggccaccaccatgttgatccagcccatggcagcagaggcagcctcctagcgtcctggctgggcctggtcccaggcccacgaaagacggtgactcttggctctgcccgaggatgtggccgttccctgcctgggcaggggctccaaggaggggccatctggaaacttgtggacagagaagaagaccacgactggagaagccccctttctgagtgcaggggggctgcatgcgttgcctcctgagatcgaggctgcaggatatgctcagactctagaggcgtggaccaaggggcatggagcttcactccttgctggccagggagttggggactcagagggaccacttggggccagccagactggcctcaatggcggactcagtcacattgactgacggggaccagggcttgtgtgggtcgagagcgccctcatggtgctggtgctgttgtgtgtaggtcccctggggacacaagcaggcgccaatggtatctgggcggagctcacagagttcttggaataaaagcaacctcagaacacttaaaaaaaaaaaaaaaaaaaaaaaaaaaaaaaaaaaaaaaaaaaaaaaaaaaaaaaaaaaaaaaa

SEQ ID NO: 5 - protein, 405 aa, Rattus norvegicus
MRCAPTAGAALVLCAATAGLLSAQGRPAQPEPPRFASWDEMNLLAHGLLQLGHGLREHVERTRGQLGALERRMAACGNACQGPKGTDPKDRVPEGQAPETLQSLQTQLKAQNSKIQQLFQKVAQQQRYLSKQNLRIQNLQSQIDLLTPTHLDNGVDKTSRGKRLPKMAQLIGLTPNATRLHRPPRDCQELFQEGERHSGLFQIQPLGSPPFLVNCEMTSDGGWTVIQRRLNGSVDFNQSWEAYKDGFGDPQGEFWLGLEKMHSITGDRGSQLAVQLQDWDGNAKLLQFPIHLGGEDTAYSLQLTEPTANELGATNVSPNGLSLPFSTWDQDHDLRGDLNCAKSLSGGWWFGTCSHSNLNGQYFHSIPRQRQQRKKGIFWKTWKGRYYPLQATTLLIQPMEATAAS

SEQ ID NO: 6 - DNA, 1218 bp, Rattus norvegicus
atgcgctgcgctccgaccgcaggcgctgctctagtgctatgcgcagctactgcggggctgctgagcgcgcaagggcgccctgcacagccggagccgccgcgcttcgcatcctgggatgaaatgaacttgctggctcacgggctgctgcagctcggtcacgggctgcgggaacacgtggagcgcacccgtggacagctgggcgcgctggaacgccgcatggctgcctgcggtaacgcttgtcaggggcccaaggggacagacccgaaggatagagtccccgaaggccaggctcctgagactctgcagagtttacagactcaactcaaggctcagaacagcaagatccagcaactgttccagaaggtagcccagcagcagagatacctatcaaagcagaatctgagaatacagaatcttcagagccagattgacctcttgacccccacacacctagacaatggggtagacaagacttcgaggggaaagaggcttcccaagatggcccagctcattggcttgactcccaacgccacccgcttacacaggcctccccgggactgccaggaactctttcaagaaggggagcggcacagtggacttttccagatccagcctctgggatctccaccatttttggtcaactgtgagatgacttcagatggaggctggacggtgattcagagacgcctgaacggctctgtggacttcaatcagtcttgggaagcctacaaagatggcttcggagatccccaaggcgagttctggctgggcctagagaagatgcacagcatcacaggggaccgaggaagccagttggctgtgcagctccaggactgggatggcaatgccaaattgctccaatttcctatccatttggggggtgaggacacagcctacagcctgcagctcaccgagcccacggccaatgagctgggtgccaccaatgtttcccccaatggcctttccctgcccttctctacctgggaccaagaccacgacctccgaggggaccttaactgtgccaagagcctctctggtggctggtggtttggcacctgcagccattccaatctaaatggacaatacttccactctattccacggcaacggcagcagcgtaaaaaggggatcttctggaaaacatggaagggccgctactatccactacaggctaccaccctgttgatccagcccatggaggctacagcagcctcttag

SEQ ID NO: 7 - protein, 410 aa, Mus musculus
MRCAPTAGAALVLCAATAGLLSAQGRPAQPEPPRFASWDEMNLLAHGLLQLGHGLREHVERTRGQLGALERRMAACGNACQGPKGKDAPFKDSEDRVPEGQTPETLQSLQTQLKAQNSKIQQLFQKVAQQQRYLSKQNLRIQNLQSQIDLLAPTHLDNGVDKTSRGKRLPKMTQLIGLTPNATHLHRPPRDCQELFQEGERHSGLFQIQPLGSPPFLVNCEMTSDGGWTVIQRRLNGSVDFNQSWEAYKDGFGDPQGEFWLGLEKMHSITGNRGSQLAVQLQDWDGNAKLLQFPIHLGGEDTAYSLQLTEPTANELGATNVSPNGLSLPFSTWDQDHDLRGDLNCAKSLSGGWWFGTCSHSNLNGQYFHSIPRQRQERKKGIFWKTWKGRYYPLQATTLLIQPMEATAAS

SEQ ID NO: 8 - DNA, 1869 bp, Mus musculus
acgggctccagatcttcttctgcaccagagcaagtctaagtctgagccggctcccccagaactccagctgctgggtcttgaactcctgcgttccggagtcctagcgttgctgcacccaaggccacccccagaatcatgcgctgcgctccgacagcaggcgctgccctggtgctatgcgcggctactgcggggcttttgagcgcgcaagggcgccctgcacagccagagccaccgcgctttgcatcctgggacgagatgaacttgctggctcacgggctgctacagctcggccatgggctgcgcgaacacgtggagcgcacccgtgggcagctgggcgcgctggagcgccgcatggctgcctgtggtaacgcttgtcaggggcccaagggaaaagatgcacccttcaaagactccgaggatagagtccctgaaggccagactcctgagactctgcagagtttgcagactcagctcaaggctcaaaacagcaagatccagcaattgttccagaaggtggcccagcagcagagatacctatcaaagcagaatctgagaatacagaatcttcagagccagatagacctcttggcccccacgcacctagacaatggagtagacaagacttcgaggggaaagaggcttcccaagatgacccagctcattggcttgactcccaacgccacccacttacacaggccgccccgggactgccaggaactcttccaagaaggggagaggcacagtggacttttccagatccagcctctggggtctccaccatttttggtcaactgtgagatgacttcagatggaggctggacagtgattcagagacgcctgaacggctctgtggacttcaaccagtcctgggaagcctacaaggatggcttcggagatccccaaggcgagttctggctgggcctggaaaagatgcacagcatcacagggaaccgaggaagccaattggctgtgcagctccaggactgggatggcaatgccaaattgctccaatttcccatccatttggggggtgaggacacagcctacagcctgcagctcactgagcccacggccaatgagctgggtgccaccaatgtttcccccaatggcctttccctgcccttctctacttgggaccaagaccatgacctccgtggggaccttaactgtgccaagagcctctctggtggctggtggtttggtacctgtagccattccaatctcaatggacaatacttccactctatcccacggcaacggcaggagcgtaaaaagggtatcttctggaaaacatggaagggccgctactatcctctgcaggctaccaccctgctgatccagcccatggaggctacagcagcctcttagcctcctcactggagcctggttccaggcctaagaagacagtgactttggttgtggccctgagatttggccattctctgctgggggcaggagctctaagtagggctatctgcgtcttgtggacaaagaagaagcccgtaactggagagactggaggaccccttttccgtgttggggtctgcaagcattgttgtctgaaacagtcagagcaacaggaaacaaatggcccagatccagaaaacatgggctcgaggggcactgaatatcacttctcgcctaccagagaagttggggatgcagagggaccactacagtccaactagctgggcccttaatggcggactcagtcatattgactgactggagacagggtgccaggagccctggatacactcatggtgctgttgtaggtgctgtggatgcacaggtgctaactgtggttcccaggcacaactcacagcattcttacaataaaaacaacctcagaacaaaaaaaaaaaaaaa

SEQ ID NO: 9 - protein, 406 aa, Homo sapiens
  MISC_FEATURE (39)..(39): x = A, K, E or D
  MISC_FEATURE (40)..(40): x = A, K, E or D
  MISC_FEATURE (76)..(76): x = C, A or S
  MISC_FEATURE (80)..(80): x = C, A or S
  MISC_FEATURE (161)..(161): x = D, R, K, G, A, V or S
  MISC_FEATURE (162)..(162): x = D, R, K, G, A, V or S
  MISC_FEATURE (163)..(163): x = D, R, K, G, A, V or S
  MISC_FEATURE (164)..(164): x = D, R, K, G, A, V or S
  misc_feature (221)..(221): Xaa can be any naturally occurring amino acid
MSGAPTAGAALMLCAATAVLLSAQGGPVQSKSPRFASWXXMNVLAHGLLQLGQGLREHAERTRSQLSALERRLSAXGSAXQGTEGSTDLPLAPESRVDPEVLHSLQTQLKAQNSRIQQLFHKVAQQQRHLEKQHLRIQHLQSQFGLLDHKHLDHEVAKPAXXXXLPEMAQPVDPAHNVSRLHRLPRDCQELFQVGERQSGLFEIQPQGSPPFLVNCKMTSXGGWTVIQRRHDGSVDFNRPWEAYKAGFGDPHGEFWLGLEKVHSITGDRNSRLAVQLRDWDGNAELLQFSVHLGGEDTAYSLQLTAPVAGQLGATTVPPSGLSVPFSTWDQDHDLRRDKNCAKSLSGGWWFGTCSHSNLNGQYFRSIPQQRQKLKKGIFWKTWRGRYYPLQATTMLIQPMAAEAAS

SEQ ID NO: 10 - protein, 368 aa, Homo sapiens
  MISC_FEATURE (39)..(39): x = A, K, D or E
  MISC_FEATURE (40)..(40): x = A, K, D or E
  MISC_FEATURE (76)..(76): x = C, A or C
  MISC_FEATURE (80)..(80): x = S, A or C
  MISC_FEATURE (161)..(161): x = D, R, K, G, A, V or S
  MISC_FEATURE (162)..(162): x = D, R, K, G, A, V or S
  MISC_FEATURE (163)..(163): x = D, R, K, G, A, V or S
  MISC_FEATURE (164)..(164): x = D, R, K, G, A, V or S
MSGAPTAGAALMLCAATAVLLSAQGGPVQSKSPRFASWXXMNVLAHGLLQLGQGLREHAERTRSQLSALERRLSAXGSAXQGTEGSTDLPLAPESRVDPEVLHSLQTQLKAQNSRIQQLFHKVAQQQRHLEKQHLRIQHLQSQFGLLDHKHLDHEVAKPAXXXXLPEMAQPVDPAHNVSRLHHGGWTVIQRRHDGSVDFNRPWEAYKAGFGDPHGEFWLGLEKVHSITGDRNSRLAVQLRDWDGNAELLQFSVHLGGEDTAYSLQLTAPVAGQLGATTVPPSGLSVPFSTWDQDHDLRRDKNCAKSLSGGWWFGTCSHSNLNGQYFRSIPQQRQKLKKGIFWKTWRGRYYPLQATTMLIQPMAAEAAS

SEQ ID NO: 11 - DNA, 22 bp, Artificial Sequence
  PCR Primer
tctgggatctccaccatttttg

SEQ ID NO: 12 - DNA, 18 bp, Artificial Sequence
  PCR Primer
tcaccgtccagcctccat

SEQ ID NO: 13 - DNA, 18 bp, Artificial Sequence
  Probe
caactgtgagatgacttc

SEQ ID NO: 14 - DNA, 17 bp, Artificial Sequence
  PCR Primer
cgccacccgcttacaca

SEQ ID NO: 15 - DNA, 22 bp, Artificial Sequence
  PCR Primer
cagaggctggatctggaaaagt

SEQ ID NO: 16 - DNA, 15 bp, Artificial Sequence
  Probe
tgccaggaactcttt

SEQ ID NO: 17 - DNA, 23 bp, Artificial Sequence
  PCR Primer
tacaggctaccaccctgttgatc

SEQ ID NO: 18 - DNA, 17 bp, Artificial Sequence
  PCR Primer
aaccgcgggccctctag

SEQ ID NO: 19 - DNA, 17 bp, Artificial Sequence
  PCR Primer
ccatggaggctacagca

SEQ ID NO: 20 - DNA, 27 bp, Artificial Sequence
  PCR Primer
cttgaagggattgaaaagataattagc

SEQ ID NO: 21 - DNA, 24 bp, Artificial Sequence
  PCR Primer
ccatgagtcagaaaagcattgaac

SEQ ID NO: 22 - DNA, 17 bp, Artificial Sequence
  Probe
aggtgagcattttcctg

SEQ ID NO: 23 - protein, 98 aa, Homo sapiens
  misc_feature (2)..(3): Xaa can be any naturally occurring amino acid
  misc_feature (5)..(5): Xaa can be any naturally occurring amino acid
  misc_feature (12)..(12): Xaa can be any naturally occurring amino acid
  misc_feature (19)..(19): Xaa can be any naturally occurring amino acid
  misc_feature (26)..(26): Xaa can be any naturally occurring amino acid
  misc_feature (28)..(28): Xaa can be any naturally occurring amino acid
  misc_feature (30)..(32): Xaa can be any naturally occurring amino acid
  misc_feature (39)..(55): Xaa can be any naturally occurring amino acid
  misc_feature (59)..(59): Xaa can be any naturally occurring amino acid
  misc_feature (64)..(64): Xaa can be any naturally occurring amino acid
  misc_feature (67)..(67): Xaa can be any naturally occurring amino acid
  misc_feature (72)..(74): Xaa can be any naturally occurring amino acid
  misc_feature (76)..(78): Xaa can be any naturally occurring amino acid
  misc_feature (80)..(80): Xaa can be any naturally occurring amino acid
  misc_feature (83)..(84): Xaa can be any naturally occurring amino acid
  misc_feature (86)..(98): Xaa can be any naturally occurring amino acid
MXXAXTAGAALXLCAATAXLLSAQGXPXQXXXPRFASWXXXXXXXXXXXXXXXXXREHXERTRXQLXALERXXXAXXXAXQGXXGXXXXXXXXXXXXX

SEQ ID NO: 24 - protein, 85 aa, Homo sapiens
  misc_feature (3)..(3): Xaa can be any naturally occurring amino acid
  misc_feature (5)..(5): Xaa can be any naturally occurring amino acid
  misc_feature (17)..(17): Xaa can be any naturally occurring amino acid
  misc_feature (23)..(23): Xaa can be any naturally occurring amino acid
  misc_feature (31)..(31): Xaa can be any naturally occurring amino acid
  misc_feature (33)..(33): Xaa can be any naturally occurring amino acid
  misc_feature (36)..(36): Xaa can be any naturally occurring amino acid
  misc_feature (41)..(41): Xaa can be any naturally occurring amino acid
  misc_feature (46)..(47): Xaa can be any naturally occurring amino acid
  misc_feature (50)..(52): Xaa can be any naturally occurring amino acid
  misc_feature (56)..(57): Xaa can be any naturally occurring amino acid
  misc_feature (59)..(59): Xaa can be any naturally occurring amino acid
  misc_feature (61)..(66): Xaa can be any naturally occurring amino acid
  misc_feature (69)..(69): Xaa can be any naturally occurring amino acid
  misc_feature (71)..(71): Xaa can be any naturally occurring amino acid
  misc_feature (73)..(78): Xaa can be any naturally occurring amino acid
  misc_feature (80)..(82): Xaa can be any naturally occurring amino acid
  misc_feature (85)..(85): Xaa can be any naturally occurring amino acid
PEXLXSLQTQLKAQNSXIQQLFXKVAQQQRXLXKQXLRIQXLQSQXXLLXXXHLDXXVXKXXXXXXLPXMXQXXXXXXNXXXLHX

SEQ ID NO: 25 - protein, 185 aa, Homo sapiens
  misc_feature (9)..(12): Xaa can be any naturally occurring amino acid
  misc_feature (16)..(16): Xaa can be any naturally occurring amino acid
  misc_feature (18)..(19): Xaa can be any naturally occurring amino acid
  misc_feature (25)..(25): Xaa can be any naturally occurring amino acid
  misc_feature (30)..(31): Xaa can be any naturally occurring amino acid
  misc_feature (41)..(41): Xaa can be any naturally occurring amino acid
  misc_feature (45)..(45): Xaa can be any naturally occurring amino acid
  misc_feature (47)..(47): Xaa can be any naturally occurring amino acid
  misc_feature (49)..(49): Xaa can be any naturally occurring amino acid
  misc_feature (51)..(51): Xaa can be any naturally occurring amino acid
  misc_feature (57)..(57): Xaa can be any naturally occurring amino acid
  misc_feature (64)..(64): Xaa can be any naturally occurring amino acid
  misc_feature (69)..(70): Xaa can be any naturally occurring amino acid
  misc_feature (72)..(72): Xaa can be any naturally occurring amino acid
  misc_feature (75)..(75): Xaa can be any naturally occurring amino acid
  misc_feature (85)..(87): Xaa can be any naturally occurring amino acid
  misc_feature (89)..(90): Xaa can be any naturally occurring amino acid
  misc_feature (95)..(95): Xaa can be any naturally occurring amino acid
  misc_feature (97)..(97): Xaa can be any naturally occurring amino acid
  misc_feature (99)..(99): Xaa can be any naturally occurring amino acid
  misc_feature (103)..(103): Xaa can be any naturally occurring amino acid
  misc_feature (115)..(118): Xaa can be any naturally occurring amino acid
  misc_feature (128)..(128): Xaa can be any naturally occurring amino acid
  misc_feature (140)..(140): Xaa can be any naturally occurring amino acid
  misc_feature (144)..(144): Xaa can be any naturally occurring amino acid
  misc_feature (148)..(148): Xaa can be any naturally occurring amino acid
  misc_feature (150)..(150): Xaa can be any naturally occurring amino acid
  misc_feature (152)..(153): Xaa can be any naturally occurring amino acid
  misc_feature (163)..(163): Xaa can be any naturally occurring amino acid
  misc_feature (174)..(174): Xaa can be any naturally occurring amino acid
  misc_feature (180)..(180): Xaa can be any naturally occurring amino acid
  misc_feature (182)..(182): Xaa can be any naturally occurring amino acid
GGWTVIQRXXXXSVDXNXXWEAYKXGFGDXXGEFWLGLEKXHSIXGXRXSXLAVQLXDWDGNAXLLQFXXHXGGXDTAYSLQLTXXXAXXLGATXVXPXGLSXPFSTWDQDHDLXXXXNCAKSLSGGXWFGTCSHSNLNXQYFXSIPXQXQXXKKGIFWKTWXGRYYPLQATTXLIQPMXAXAAS

SEQ ID NO: 26 - protein, 183 aa, Homo sapiens
  misc_feature (5)..(5): Xaa can be any naturally occurring amino acid
  MISC_FEATURE (39)..(55): Anti-LPL activity region
  misc_feature (67)..(67): Xaa can be any naturally occurring amino acid
  misc_feature (72)..(72): Xaa can be any naturally occurring amino acid
  misc_feature (76)..(77): Xaa can be any naturally occurring amino acid
  misc_feature (80)..(80): Xaa can be any naturally occurring amino acid
  MISC_FEATURE (161)..(164): Cleavage region
  misc_feature (167)..(167): Xaa can be any naturally occurring amino acid
  misc_feature (174)..(174): Xaa can be any naturally occurring amino acid
  misc_feature (183)..(183): Xaa can be any naturally occurring amino acid
MSGAXTAGAALMLCAATAVLLSAQGGPVQSKSPRFASWXXXXXXXXXXXXXXXXXREHAERTRSQLXALERXLSAXXSAXQGTEGSTDLPLAPESRVDPEVLHSLQTQLKAQNSRIQQLFHKVAQQQRHLEKQHLRIQHLQSQFGLLDHKHLDHEVAKPAXXXXLPXMAQPVDXAHNVSRLHX

SEQ ID NO: 27 - protein, 185 aa, Homo sapiens
  misc_feature (9)..(9): Xaa can be any naturally occurring amino acid
  misc_feature (12)..(12): Xaa can be any naturally occurring amino acid
  misc_feature (16)..(16): Xaa can be any naturally occurring amino acid
  misc_feature (30)..(30): Xaa can be any naturally occurring amino acid
  misc_feature (45)..(45): Xaa can be any naturally occurring amino acid
  misc_feature (57)..(57): Xaa can be any naturally occurring amino acid
  misc_feature (70)..(70): Xaa can be any naturally occurring amino acid
  misc_feature (72)..(72): Xaa can be any naturally occurring amino acid
  misc_feature (75)..(75): Xaa can be any naturally occurring amino acid
  misc_feature (86)..(87): Xaa can be any naturally occurring amino acid
  misc_feature (115)..(115): Xaa can be any naturally occurring amino acid
  misc_feature (117)..(117): Xaa can be any naturally occurring amino acid
  misc_feature (128)..(128): Xaa can be any naturally occurring amino acid
  misc_feature (140)..(140): Xaa can be any naturally occurring amino acid
  misc_feature (150)..(150): Xaa can be any naturally occurring amino acid
  misc_feature (163)..(163): Xaa can be any naturally occurring amino acid
GGWTVIQRXHDXSVDXNRPWEAYKAGFGDXHGEFWLGLEKVHSIXGDRNSRLAVQLXDWDGNAELLQFSXHXGGXDTAYSLQLTAXXAGQLGATTVPPSGLSVPFSTWDQDHDLXRXKNCAKSLSGGXWFGTCSHSNLNXQYFRSIPQQXQKLKKGIFWKTWXGRYYPLQATTMLIQPMAAEAAS

SEQ ID NO: 28 - protein, 17 aa, Homo sapiens
DKMNVLAHGLLQLGQGL

SEQ ID NO: 29 - protein, 4 aa, Artificial Sequence
  Mutations at postitions 161-164
GAAG

SEQ ID NO: 30 - protein, 4 aa, Artificial Sequence
  Mutations at postitions 161-164
GAGA

SEQ ID NO: 31 - protein, 4 aa, Artificial Sequence
  Mutations at postitions 161-164
GGAA

SEQ ID NO: 32 - protein, 4 aa, Artificial Sequence
  Mutations at postitions 161-164
AGGA

SEQ ID NO: 33 - protein, 4 aa, Artificial Sequence
  Mutations at postitions 161-164
AGAG

SEQ ID NO: 34 - protein, 4 aa, Artificial Sequence
  Mutations at postitions 161-164
AAGG

SEQ ID NO: 35 - protein, 4 aa, Artificial Sequence
  Mutations at postitions 161-164
VGAA

SEQ ID NO: 36 - protein, 4 aa, Artificial Sequence
  Mutations at postitions 161-164
VAAG

SEQ ID NO: 37 - protein, 4 aa, Artificial Sequence
  Mutations at postitions 161-164
VAGA

SEQ ID NO: 38 - protein, 4 aa, Artificial Sequence
  Mutations at postitions 161-164
GAAV

SEQ ID NO: 39 - protein, 4 aa, Artificial Sequence
  Mutations at postitions 161-164
GAVA

SEQ ID NO: 40 - protein, 4 aa, Artificial Sequence
  Mutations at postitions 161-164
GVAA

SEQ ID NO: 41 - protein, 4 aa, Artificial Sequence
  Mutations at postitions 161-164
AGVA

SEQ ID NO: 42 - protein, 4 aa, Artificial Sequence
  Mutations at postitions 161-164
AGAV

SEQ ID NO: 43 - protein, 4 aa, Artificial Sequence
  Mutations at postitions 161-164
AAVG

SEQ ID NO: 44 - protein, 4 aa, Artificial Sequence
  Mutations at postitions 161-164
AAGV

SEQ ID NO: 45 - protein, 4 aa, Artificial Sequence
  Mutations at postitions 161-164
AVAG

SEQ ID NO: 46 - protein, 4 aa, Artificial Sequence
  Mutations at postitions 161-164
AVGA

SEQ ID NO: 47 - protein, 4 aa, Artificial Sequence
  Mutations at postitions 161-164
GAVV

SEQ ID NO: 48 - protein, 4 aa, Artificial Sequence
  Mutations at postitions 161-164
GVAV

SEQ ID NO: 49 - protein, 4 aa, Artificial Sequence
  Mutations at postitions 161-164
GVVA

SEQ ID NO: 50 - protein, 4 aa, Artificial Sequence
  Mutations at postitions 161-164
AGVV

SEQ ID NO: 51 - protein, 4 aa, Artificial Sequence
  Mutations at postitions 161-164
AVVG

SEQ ID NO: 52 - protein, 4 aa, Artificial Sequence
  Mutations at postitions 161-164
AVGV

SEQ ID NO: 53 - protein, 4 aa, Artificial Sequence
  Mutations at postitions 161-164
VGAV

SEQ ID NO: 54 - protein, 4 aa, Artificial Sequence
  Mutations at postitions 161-164
VGVA

SEQ ID NO: 55 - protein, 4 aa, Artificial Sequence
  Mutations at postitions 161-164
VAGV

SEQ ID NO: 56 - protein, 4 aa, Artificial Sequence
  Mutations at postitions 161-164
GVVV

SEQ ID NO: 57 - protein, 4 aa, Artificial Sequence
  Mutations at postitions 161-164
VGVV

SEQ ID NO: 58 - protein, 4 aa, Artificial Sequence
  Mutations at postitions 161-164
VVVG

SEQ ID NO: 59 - protein, 4 aa, Artificial Sequence
  Mutations at postitions 161-164
VVGV

SEQ ID NO: 60 - protein, 4 aa, Artificial Sequence
  Mutations at postitions 161-164
VAVG

SEQ ID NO: 61 - protein, 4 aa, Artificial Sequence
  Mutations at postitions 161-164
VVGA

SEQ ID NO: 62 - protein, 4 aa, Artificial Sequence
  Mutations at postitions 161-164
VVAG

SEQ ID NO: 63 - protein, 4 aa, Artificial Sequence
  Mutations at postitions 161-164
VVVA

SEQ ID NO: 64 - protein, 4 aa, Artificial Sequence
  Mutations at postitions 161-164
VVAV

SEQ ID NO: 65 - protein, 4 aa, Artificial Sequence
  Mutations at postitions 161-164
GAAA

SEQ ID NO: 66 - protein, 4 aa, Artificial Sequence
  Mutations at postitions 161-164
AGAA

SEQ ID NO: 67 - protein, 4 aa, Artificial Sequence
  Mutations at postitions 161-164
AAAG

SEQ ID NO: 68 - protein, 4 aa, Artificial Sequence
  Mutations at postitions 161-164
AAGA

SEQ ID NO: 69 - protein, 4 aa, Artificial Sequence
  Mutations at postitions 161-164
AAVV

SEQ ID NO: 70 - protein, 4 aa, Artificial Sequence
  Mutations at postitions 161-164
AAVA

SEQ ID NO: 71 - protein, 4 aa, Artificial Sequence
  Mutations at postitions 161-164
AAAV

SEQ ID NO: 72 - protein, 4 aa, Artificial Sequence
  Mutations at postitions 161-164
AVAA

SEQ ID NO: 73 - protein, 4 aa, Artificial Sequence
  Mutations at postitions 161-164
VAAA

SEQ ID NO: 74 - protein, 4 aa, Artificial Sequence
  Mutations at postitions 161-164
AVVV

SEQ ID NO: 75 - protein, 4 aa, Artificial Sequence
  Mutations at postitions 161-164
VAVV

SEQ ID NO: 76 - protein, 4 aa, Artificial Sequence
  Mutations at postitions 161-164
VVVV

SEQ ID NO: 77 - protein, 4 aa, Artificial Sequence
  Mutations at postitions 161-164
SSSS

SEQ ID NO: 78 - protein, 4 aa, Artificial Sequence
  Mutations at postitions 161-164
GGGG

SEQ ID NO: 79 - protein, 4 aa, Artificial Sequence
  Mutations at postitions 161-164
AAAA

SEQ ID NO: 80 - protein, 4 aa, Artificial Sequence
  Mutations at postitions 161-164
GSGS

SEQ ID NO: 81 - protein, 4 aa, Artificial Sequence
  Mutations at postitions 161-164
GSSG

SEQ ID NO: 82 - protein, 4 aa, Artificial Sequence
  Mutations at postitions 161-164
GGSS

SEQ ID NO: 83 - protein, 4 aa, Artificial Sequence
  Mutations at postitions 161-164
SGSG

SEQ ID NO: 84 - protein, 4 aa, Artificial Sequence
  Mutations at postitions 161-164
SGGS

SEQ ID NO: 85 - protein, 4 aa, Artificial Sequence
  Mutations at postitions 161-164
SSGG

SEQ ID NO: 86 - protein, 4 aa, Artificial Sequence
  Mutations at postitions 161-164
GSGG

SEQ ID NO: 87 - protein, 4 aa, Artificial Sequence
  Mutations at postitions 161-164
SGGG

SEQ ID NO: 88 - protein, 4 aa, Artificial Sequence
  Mutations at postitions 161-164
GGSG

SEQ ID NO: 89 - protein, 4 aa, Artificial Sequence
  Mutations at postitions 161-164
GGGS

SEQ ID NO: 90 - protein, 4 aa, Artificial Sequence
  Mutations at postitions 161-164
VAVA

SEQ ID NO: 91 - DNA, 23 bp, Artificial Sequence
  PCR Primer
agggataggcttaccttcgaatg

SEQ ID NO: 92 - DNA, 12 bp, Artificial Sequence
  Probe
cagcagcctccc

SEQ ID NO: 93 - DNA, 16 bp, Artificial Sequence
  mutant Angptl4 8501 cDNA
ccggatcaggatcact

SEQ ID NO: 94 - DNA, 16 bp, Artificial Sequence
  mutant Angptl4 8515 cDNA
cctccggcggcggcct